European Patent Application EP 4 674 869 A1, published January 7, 2026. Title: Method for treatment of advanced or metastatic solid cancer using anti-CD47 antibody. Applicant: ImmuneOncia Therapeutics Inc. Application KR, filed October 15, 2024. The sequence listing filed with the application follows.

SEQUENCE LISTING (10 sequences)

SEQ ID NO: 1 - protein, 119 aa, Artificial Sequence
QVQLVQSGAEVKKPGASVKVSCKASGYTFTSYYMHWVRQAPGQGLEWMGIINPSGGSTSYAQKFQGRVTMTRDTSTSTVYMELSSLRSEDTAVYYCARSTLWVSEFDYWGQGTLVTVSS

SEQ ID NO: 2 - protein, 110 aa, Artificial Sequence
QSALTQPASVSGSPGQSISISCTGTSSDVGGHNYVSWYQQHPGKAPKLMIYDVRNRPSGVSNRFSGSKSGSTASLTISGLQTEDEADYYCNSYTGSRTYVFGSGTKLTVL

SEQ ID NO: 3 - protein, 446 aa, Artificial Sequence
QVQLVQSGAEVKKPGASVKVSCKASGYTFTSYYMHWVRQAPGQGLEWMGIINPSGGSTSYAQKFQGRVTMTRDTSTSTVYMELSSLRSEDTAVYYCARSTLWVSEFDYWGQGTLVTVSSASTKGPSVFPLAPCSRSTSESTAALGCLVKDYFPEPVTVSWNSGALTSGVHTFPAVLQSSGLYSLSSVVTVPSSSLGTKTYTCNVDHKPSNTKVDKRVESKYGPPCPPCPAPEFLGGPSVFLFPPKPKDTLMISRTPEVTCVVVDVSQEDPEVQFNWYVDGVEVHNAKTKPREEQFNSTYRVVSVLTVLHQDWLNGKEYKCKVSNKGLPSSIEKTISKAKGQPREPQVYTLPPSQEEMTKNQVSLTCLVKGFYPSDIAVEWESNGQPENNYKTTPPVLDSDGSFFLYSRLTVDKSRWQEGNVFSCSVMHEALHNHYTQKSLSLSLGK

SEQ ID NO: 4 - protein, 216 aa, Artificial Sequence
QSALTQPASVSGSPGQSISISCTGTSSDVGGHNYVSWYQQHPGKAPKLMIYDVRNRPSGVSNRFSGSKSGSTASLTISGLQTEDEADYYCNSYTGSRTYVFGSGTKLTVLGQPKAAPSVTLFPPSSEELQANKATLVCLISDFYPGAVTVAWKADSSPVKAGVETTTPSKQSNNKYAASSYLSLTPEQWKSHRSYSCQVTHEGSTVEKTVAPTECS

SEQ ID NO: 5 - protein, 7 aa, Artificial Sequence
GYTFTSY

SEQ ID NO: 6 - protein, 6 aa, Artificial Sequence
NPSGGS

SEQ ID NO: 7 - protein, 10 aa, Artificial Sequence
STLWVSEFDY

SEQ ID NO: 8 - protein, 14 aa, Artificial Sequence
TGTSSDVGGHNYVS

SEQ ID NO: 9 - protein, 7 aa, Artificial Sequence
DVRNRPS

SEQ ID NO: 10 - protein, 10 aa, Artificial Sequence
NSYTGSRTYV